European Patent Specification EP 4 023 663 B1, published February 26, 2025. Title: Polypeptide and application thereof. Applicant: HDL SOLUTIONS OTTAWA. Application EP20855987.2. The sequence listing filed with the application follows.

SEQUENCE LISTING (8 sequences)

SEQ ID NO: 1 - protein, 23 aa, Artificial Sequence
  polypeptide
FAYLQDVVEQAIIRVLTGTEKKT

SEQ ID NO: 2 - protein, 22 aa, Artificial Sequence
  polypeptide
FAYLQDVVEQAIIRVLTGTEKK

SEQ ID NO: 3 - protein, 21 aa, Artificial Sequence
  polypeptide
FAYLQDVVEQAIIRVLTGTEK

SEQ ID NO: 4 - protein, 20 aa, Artificial Sequence
  polypeptide
FAYLQDVVEQAIIRVLTGTE

SEQ ID NO: 5 - protein, 19 aa, Artificial Sequence
  polypeptide
FAYLQDVVEQAIIRVLTGT

SEQ ID NO: 6 - protein, 18 aa, Artificial Sequence
  polypeptide
FAYLQDVVEQAIIRVLTG

SEQ ID NO: 7 - protein, 17 aa, Artificial Sequence
  polypeptide
FAYLQDVVEQAIIRVLT

SEQ ID NO: 8 - protein, 16 aa, Artificial Sequence
  polypeptide
FAYLQDVVEQAIIRVL